European Patent Specification EP 3 647 785 B1, published November 20, 2024. Title: A Method for Measuring Serum Amyloid A of Various Animals and A Measurement Reagent Thereof. Applicant: Eiken Kagaku Kabushiki Kaisha. The sequence listing filed with the application follows.

SEQUENCE LISTING (14 sequences)

SEQ ID NO: 1 - protein, 104 aa, Homo sapiens
RSFFSFLGEAFDGARDMWRAYSDMREANYIGSDKYFHARGNYDAAKRGPGGVWAAEAISDARENIQRFFGHGAEDSLADQAANEWGRSGKDPNHFRPAGLPEKY

SEQ ID NO: 2 - protein, 25 aa, Artificial
  synthetic
HGAEDSLADQAANEWGRSGKDPNHF

SEQ ID NO: 3 - protein, 15 aa, Artificial
  synthetic
HGAEDSLADQAANEW

SEQ ID NO: 4 - protein, 15 aa, Artificial
  synthetic
GAEDSLADQAANEWG

SEQ ID NO: 5 - protein, 15 aa, Artificial
  synthetic
AEDSLADQAANEWGR

SEQ ID NO: 6 - protein, 15 aa, Artificial
  synthetic
EDSLADQAANEWGRS

SEQ ID NO: 7 - protein, 15 aa, Artificial
  synthetic
DSLADQAANEWGRSG

SEQ ID NO: 8 - protein, 15 aa, Artificial
  synthetic
SLADQAANEWGRSGK

SEQ ID NO: 9 - protein, 15 aa, Artificial
  synthetic
LADQAANEWGRSGKD

SEQ ID NO: 10 - protein, 15 aa, Artificial
  synthetic
ADQAANEWGRSGKDP

SEQ ID NO: 11 - protein, 15 aa, Artificial
  synthetic
DQAANEWGRSGKDPN

SEQ ID NO: 12 - protein, 15 aa, Artificial
  synthetic
QAANEWGRSGKDPNH

SEQ ID NO: 13 - protein, 15 aa, Artificial
  synthetic
AANEWGRSGKDPNHF

SEQ ID NO: 14 - protein, 11 aa, Homo sapiens
QAANEWGRSGK